European Patent Specification EP 4 114 865 B1, published January 28, 2026. Title: Protease-Processed Molecules. Applicant: SANOFI. The sequence listing filed with the application follows.

SEQUENCE LISTING (75 sequences)

SEQ ID NO: 1 - protein, 724 aa, Artificial Sequence
  anti-IL4-VL-huIGKC-[PCS1]-<(G4S)10>-[PCS1]-anti-IL4-VH-huIGHG1
DIQMTQSPASLSVSVGDTITLTCHASQNIDVWLSWFQQKPGNIPKLLIYKASNLHTGVPSRFSGSGSGTGFTLTISSLQPEDIATYYCQQAHSYPFTFGGGTKLEIKRTVAAPSVFIFPPSDEQLKSGTASVVCLLNNFYPREAKVQWKVDNALQSGNSQESVTEQDSKDSTYSLSSTLTLSKADYEKHKVYACEVTHQGLSSPVTKSFNRGECRRKRGGGGSGGGGSGGGGSGGGGSGGGGSGGGGSGGGGSGGGGSGGGGSGGGGSRRKRQVQLQQSGPELVKPGASVKISCKASGYSFTSYWIHWIKQRPGQGLEWIGMIDPSDGETRLNQRFQGRATLTVDESTSTAYMQLRSPTSEDSAVYYCTRLKEYGNYDSFYFDVWGAGTLVTVSSASTKGPSVFPLAPSSKSTSGGTAALGCLVKDYFPEPVTVSWNSGALTSGVHTFPAVLQSSGLYSLSSVVTVPSSSLGTQTYICNVNHKPSNTKVDKKVEPKSCDKTHTCPPCPAPELLGGPSVFLFPPKPKDTLMISRTPEVTCVVVDVSHEDPEVKFNWYVDGVEVHNAKTKPREEQYNSTYRVVSVLTVLHQDWLNGKEYKCKVSNKALPAPIEKTISKAKGQPREPQVYTLPPSRDELTKNQVSLTCLVKGFYPSDIAVEWESNGQPENNYKTTPPVLDSDGSFFLYSKLTVDKSRWQQGNVFSCSVMHEALHNHYTQKSLSLSPG

SEQ ID NO: 2 - protein, 714 aa, Artificial Sequence
  anti-IL4-VL-huIGKC-[PCS1]-<(G4S)8>-[PCS1]-anti-IL4-VH-huIGHG1
DIQMTQSPASLSVSVGDTITLTCHASQNIDVWLSWFQQKPGNIPKLLIYKASNLHTGVPSRFSGSGSGTGFTLTISSLQPEDIATYYCQQAHSYPFTFGGGTKLEIKRTVAAPSVFIFPPSDEQLKSGTASVVCLLNNFYPREAKVQWKVDNALQSGNSQESVTEQDSKDSTYSLSSTLTLSKADYEKHKVYACEVTHQGLSSPVTKSFNRGECRRKRGGGGSGGGGSGGGGSGGGGSGGGGSGGGGSGGGGSGGGGSRRKRQVQLQQSGPELVKPGASVKISCKASGYSFTSYWIHWIKQRPGQGLEWIGMIDPSDGETRLNQRFQGRATLTVDESTSTAYMQLRSPTSEDSAVYYCTRLKEYGNYDSFYFDVWGAGTLVTVSSASTKGPSVFPLAPSSKSTSGGTAALGCLVKDYFPEPVTVSWNSGALTSGVHTFPAVLQSSGLYSLSSVVTVPSSSLGTQTYICNVNHKPSNTKVDKKVEPKSCDKTHTCPPCPAPELLGGPSVFLFPPKPKDTLMISRTPEVTCVVVDVSHEDPEVKFNWYVDGVEVHNAKTKPREEQYNSTYRVVSVLTVLHQDWLNGKEYKCKVSNKALPAPIEKTISKAKGQPREPQVYTLPPSRDELTKNQVSLTCLVKGFYPSDIAVEWESNGQPENNYKTTPPVLDSDGSFFLYSKLTVDKSRWQQGNVFSCSVMHEALHNHYTQKSLSLSPG

SEQ ID NO: 3 - protein, 704 aa, Artificial Sequence
  anti-IL4-VL-huIGKC-[PCS1]-<(G4S)6>-[PCS1]-anti-IL4-VH-huIGHG1
DIQMTQSPASLSVSVGDTITLTCHASQNIDVWLSWFQQKPGNIPKLLIYKASNLHTGVPSRFSGSGSGTGFTLTISSLQPEDIATYYCQQAHSYPFTFGGGTKLEIKRTVAAPSVFIFPPSDEQLKSGTASVVCLLNNFYPREAKVQWKVDNALQSGNSQESVTEQDSKDSTYSLSSTLTLSKADYEKHKVYACEVTHQGLSSPVTKSFNRGECRRKRGGGGSGGGGSGGGGSGGGGSGGGGSGGGGSRRKRQVQLQQSGPELVKPGASVKISCKASGYSFTSYWIHWIKQRPGQGLEWIGMIDPSDGETRLNQRFQGRATLTVDESTSTAYMQLRSPTSEDSAVYYCTRLKEYGNYDSFYFDVWGAGTLVTVSSASTKGPSVFPLAPSSKSTSGGTAALGCLVKDYFPEPVTVSWNSGALTSGVHTFPAVLQSSGLYSLSSVVTVPSSSLGTQTYICNVNHKPSNTKVDKKVEPKSCDKTHTCPPCPAPELLGGPSVFLFPPKPKDTLMISRTPEVTCVVVDVSHEDPEVKFNWYVDGVEVHNAKTKPREEQYNSTYRVVSVLTVLHQDWLNGKEYKCKVSNKALPAPIEKTISKAKGQPREPQVYTLPPSRDELTKNQVSLTCLVKGFYPSDIAVEWESNGQPENNYKTTPPVLDSDGSFFLYSKLTVDKSRWQQGNVFSCSVMHEALHNHYTQKSLSLSPG

SEQ ID NO: 4 - protein, 694 aa, Artificial Sequence
  anti-IL4-VL-huIGKC-[PCS1]-<(G4S)4>-[PCS1]-anti-IL4-VH-huIGHG1
DIQMTQSPASLSVSVGDTITLTCHASQNIDVWLSWFQQKPGNIPKLLIYKASNLHTGVPSRFSGSGSGTGFTLTISSLQPEDIATYYCQQAHSYPFTFGGGTKLEIKRTVAAPSVFIFPPSDEQLKSGTASVVCLLNNFYPREAKVQWKVDNALQSGNSQESVTEQDSKDSTYSLSSTLTLSKADYEKHKVYACEVTHQGLSSPVTKSFNRGECRRKRGGGGSGGGGSGGGGSGGGGSRRKRQVQLQQSGPELVKPGASVKISCKASGYSFTSYWIHWIKQRPGQGLEWIGMIDPSDGETRLNQRFQGRATLTVDESTSTAYMQLRSPTSEDSAVYYCTRLKEYGNYDSFYFDVWGAGTLVTVSSASTKGPSVFPLAPSSKSTSGGTAALGCLVKDYFPEPVTVSWNSGALTSGVHTFPAVLQSSGLYSLSSVVTVPSSSLGTQTYICNVNHKPSNTKVDKKVEPKSCDKTHTCPPCPAPELLGGPSVFLFPPKPKDTLMISRTPEVTCVVVDVSHEDPEVKFNWYVDGVEVHNAKTKPREEQYNSTYRVVSVLTVLHQDWLNGKEYKCKVSNKALPAPIEKTISKAKGQPREPQVYTLPPSRDELTKNQVSLTCLVKGFYPSDIAVEWESNGQPENNYKTTPPVLDSDGSFFLYSKLTVDKSRWQQGNVFSCSVMHEALHNHYTQKSLSLSPG

SEQ ID NO: 5 - protein, 684 aa, Artificial Sequence
  anti-IL4-VL-huIGKC-[PCS1]-<(G4S)2>-[PCS1]-anti-IL4-VH-huIGHG1
DIQMTQSPASLSVSVGDTITLTCHASQNIDVWLSWFQQKPGNIPKLLIYKASNLHTGVPSRFSGSGSGTGFTLTISSLQPEDIATYYCQQAHSYPFTFGGGTKLEIKRTVAAPSVFIFPPSDEQLKSGTASVVCLLNNFYPREAKVQWKVDNALQSGNSQESVTEQDSKDSTYSLSSTLTLSKADYEKHKVYACEVTHQGLSSPVTKSFNRGECRRKRGGGGSGGGGSRRKRQVQLQQSGPELVKPGASVKISCKASGYSFTSYWIHWIKQRPGQGLEWIGMIDPSDGETRLNQRFQGRATLTVDESTSTAYMQLRSPTSEDSAVYYCTRLKEYGNYDSFYFDVWGAGTLVTVSSASTKGPSVFPLAPSSKSTSGGTAALGCLVKDYFPEPVTVSWNSGALTSGVHTFPAVLQSSGLYSLSSVVTVPSSSLGTQTYICNVNHKPSNTKVDKKVEPKSCDKTHTCPPCPAPELLGGPSVFLFPPKPKDTLMISRTPEVTCVVVDVSHEDPEVKFNWYVDGVEVHNAKTKPREEQYNSTYRVVSVLTVLHQDWLNGKEYKCKVSNKALPAPIEKTISKAKGQPREPQVYTLPPSRDELTKNQVSLTCLVKGFYPSDIAVEWESNGQPENNYKTTPPVLDSDGSFFLYSKLTVDKSRWQQGNVFSCSVMHEALHNHYTQKSLSLSPG

SEQ ID NO: 6 - protein, 724 aa, Artificial Sequence
  anti-IL4-VL-huIGKC-[deltaPCS]-<(G4S)10>-[deltaPCS]-anti-IL4-VH-huIGHG1
DIQMTQSPASLSVSVGDTITLTCHASQNIDVWLSWFQQKPGNIPKLLIYKASNLHTGVPSRFSGSGSGTGFTLTISSLQPEDIATYYCQQAHSYPFTFGGGTKLEIKRTVAAPSVFIFPPSDEQLKSGTASVVCLLNNFYPREAKVQWKVDNALQSGNSQESVTEQDSKDSTYSLSSTLTLSKADYEKHKVYACEVTHQGLSSPVTKSFNRGECRQQRGGGGSGGGGSGGGGSGGGGSGGGGSGGGGSGGGGSGGGGSGGGGSGGGGSRQQRQVQLQQSGPELVKPGASVKISCKASGYSFTSYWIHWIKQRPGQGLEWIGMIDPSDGETRLNQRFQGRATLTVDESTSTAYMQLRSPTSEDSAVYYCTRLKEYGNYDSFYFDVWGAGTLVTVSSASTKGPSVFPLAPSSKSTSGGTAALGCLVKDYFPEPVTVSWNSGALTSGVHTFPAVLQSSGLYSLSSVVTVPSSSLGTQTYICNVNHKPSNTKVDKKVEPKSCDKTHTCPPCPAPELLGGPSVFLFPPKPKDTLMISRTPEVTCVVVDVSHEDPEVKFNWYVDGVEVHNAKTKPREEQYNSTYRVVSVLTVLHQDWLNGKEYKCKVSNKALPAPIEKTISKAKGQPREPQVYTLPPSRDELTKNQVSLTCLVKGFYPSDIAVEWESNGQPENNYKTTPPVLDSDGSFFLYSKLTVDKSRWQQGNVFSCSVMHEALHNHYTQKSLSLSPG

SEQ ID NO: 7 - protein, 722 aa, Artificial Sequence
  anti-IL4-VL-huIGKC-[PCS1]-<(G4S)4>-His(8)-<(G4S)4>-[PCS1]-anti-IL4-VH-huIGHG1
DIQMTQSPASLSVSVGDTITLTCHASQNIDVWLSWFQQKPGNIPKLLIYKASNLHTGVPSRFSGSGSGTGFTLTISSLQPEDIATYYCQQAHSYPFTFGGGTKLEIKRTVAAPSVFIFPPSDEQLKSGTASVVCLLNNFYPREAKVQWKVDNALQSGNSQESVTEQDSKDSTYSLSSTLTLSKADYEKHKVYACEVTHQGLSSPVTKSFNRGECRRKRGGGGSGGGGSGGGGSGGGGSHHHHHHHHGGGGSGGGGSGGGGSGGGGSRRKRQVQLQQSGPELVKPGASVKISCKASGYSFTSYWIHWIKQRPGQGLEWIGMIDPSDGETRLNQRFQGRATLTVDESTSTAYMQLRSPTSEDSAVYYCTRLKEYGNYDSFYFDVWGAGTLVTVSSASTKGPSVFPLAPSSKSTSGGTAALGCLVKDYFPEPVTVSWNSGALTSGVHTFPAVLQSSGLYSLSSVVTVPSSSLGTQTYICNVNHKPSNTKVDKKVEPKSCDKTHTCPPCPAPELLGGPSVFLFPPKPKDTLMISRTPEVTCVVVDVSHEDPEVKFNWYVDGVEVHNAKTKPREEQYNSTYRVVSVLTVLHQDWLNGKEYKCKVSNKALPAPIEKTISKAKGQPREPQVYTLPPSRDELTKNQVSLTCLVKGFYPSDIAVEWESNGQPENNYKTTPPVLDSDGSFFLYSKLTVDKSRWQQGNVFSCSVMHEALHNHYTQKSLSLSPG

SEQ ID NO: 8 - protein, 722 aa, Artificial Sequence
  anti-IL4-VL-huIGKC-[deltaPCS]-<(G4S)4>-His(8)-<(G4S)4>-[deltaPCS]-anti-IL4-VH-huIGHG1
DIQMTQSPASLSVSVGDTITLTCHASQNIDVWLSWFQQKPGNIPKLLIYKASNLHTGVPSRFSGSGSGTGFTLTISSLQPEDIATYYCQQAHSYPFTFGGGTKLEIKRTVAAPSVFIFPPSDEQLKSGTASVVCLLNNFYPREAKVQWKVDNALQSGNSQESVTEQDSKDSTYSLSSTLTLSKADYEKHKVYACEVTHQGLSSPVTKSFNRGECRQQRGGGGSGGGGSGGGGSGGGGSHHHHHHHHGGGGSGGGGSGGGGSGGGGSRQQRQVQLQQSGPELVKPGASVKISCKASGYSFTSYWIHWIKQRPGQGLEWIGMIDPSDGETRLNQRFQGRATLTVDESTSTAYMQLRSPTSEDSAVYYCTRLKEYGNYDSFYFDVWGAGTLVTVSSASTKGPSVFPLAPSSKSTSGGTAALGCLVKDYFPEPVTVSWNSGALTSGVHTFPAVLQSSGLYSLSSVVTVPSSSLGTQTYICNVNHKPSNTKVDKKVEPKSCDKTHTCPPCPAPELLGGPSVFLFPPKPKDTLMISRTPEVTCVVVDVSHEDPEVKFNWYVDGVEVHNAKTKPREEQYNSTYRVVSVLTVLHQDWLNGKEYKCKVSNKALPAPIEKTISKAKGQPREPQVYTLPPSRDELTKNQVSLTCLVKGFYPSDIAVEWESNGQPENNYKTTPPVLDSDGSFFLYSKLTVDKSRWQQGNVFSCSVMHEALHNHYTQKSLSLSPG

SEQ ID NO: 9 - protein, 724 aa, Artificial Sequence
  anti-IL4-VL-huIGKC-[PCS2]-<(G4S)4>-His(8)-<(G4S)4>-[PCS2]-anti-IL4-VH-huIGHG1
DIQMTQSPASLSVSVGDTITLTCHASQNIDVWLSWFQQKPGNIPKLLIYKASNLHTGVPSRFSGSGSGTGFTLTISSLQPEDIATYYCQQAHSYPFTFGGGTKLEIKRTVAAPSVFIFPPSDEQLKSGTASVVCLLNNFYPREAKVQWKVDNALQSGNSQESVTEQDSKDSTYSLSSTLTLSKADYEKHKVYACEVTHQGLSSPVTKSFNRGECHRRRKRSVDEGGGGSGGGGSGGGGSHHHHHHHHGGGGSGGGGSGGGGSHRRRKRSVDEQVQLQQSGPELVKPGASVKISCKASGYSFTSYWIHWIKQRPGQGLEWIGMIDPSDGETRLNQRFQGRATLTVDESTSTAYMQLRSPTSEDSAVYYCTRLKEYGNYDSFYFDVWGAGTLVTVSSASTKGPSVFPLAPSSKSTSGGTAALGCLVKDYFPEPVTVSWNSGALTSGVHTFPAVLQSSGLYSLSSVVTVPSSSLGTQTYICNVNHKPSNTKVDKKVEPKSCDKTHTCPPCPAPELLGGPSVFLFPPKPKDTLMISRTPEVTCVVVDVSHEDPEVKFNWYVDGVEVHNAKTKPREEQYNSTYRVVSVLTVLHQDWLNGKEYKCKVSNKALPAPIEKTISKAKGQPREPQVYTLPPSRDELTKNQVSLTCLVKGFYPSDIAVEWESNGQPENNYKTTPPVLDSDGSFFLYSKLTVDKSRWQQGNVFSCSVMHEALHNHYTQKSLSLSPG

SEQ ID NO: 10 - protein, 724 aa, Artificial Sequence
  anti-IL4-VL-huIGKC-[PCS3]-<(G4S)4>-His(8)-<(G4S)4>-[PCS3]-anti-IL4-VH-huIGHG1
DIQMTQSPASLSVSVGDTITLTCHASQNIDVWLSWFQQKPGNIPKLLIYKASNLHTGVPSRFSGSGSGTGFTLTISSLQPEDIATYYCQQAHSYPFTFGGGTKLEIKRTVAAPSVFIFPPSDEQLKSGTASVVCLLNNFYPREAKVQWKVDNALQSGNSQESVTEQDSKDSTYSLSSTLTLSKADYEKHKVYACEVTHQGLSSPVTKSFNRGECPMKKRRAGVPGGGGSGGGGSGGGGSHHHHHHHHGGGGSGGGGSGGGGSPMKKRRAGVPQVQLQQSGPELVKPGASVKISCKASGYSFTSYWIHWIKQRPGQGLEWIGMIDPSDGETRLNQRFQGRATLTVDESTSTAYMQLRSPTSEDSAVYYCTRLKEYGNYDSFYFDVWGAGTLVTVSSASTKGPSVFPLAPSSKSTSGGTAALGCLVKDYFPEPVTVSWNSGALTSGVHTFPAVLQSSGLYSLSSVVTVPSSSLGTQTYICNVNHKPSNTKVDKKVEPKSCDKTHTCPPCPAPELLGGPSVFLFPPKPKDTLMISRTPEVTCVVVDVSHEDPEVKFNWYVDGVEVHNAKTKPREEQYNSTYRVVSVLTVLHQDWLNGKEYKCKVSNKALPAPIEKTISKAKGQPREPQVYTLPPSRDELTKNQVSLTCLVKGFYPSDIAVEWESNGQPENNYKTTPPVLDSDGSFFLYSKLTVDKSRWQQGNVFSCSVMHEALHNHYTQKSLSLSPG

SEQ ID NO: 11 - protein, 214 aa, Artificial Sequence
  anti-IL4-VL-huIGKC
DIQMTQSPASLSVSVGDTITLTCHASQNIDVWLSWFQQKPGNIPKLLIYKASNLHTGVPSRFSGSGSGTGFTLTISSLQPEDIATYYCQQAHSYPFTFGGGTKLEIKRTVAAPSVFIFPPSDEQLKSGTASVVCLLNNFYPREAKVQWKVDNALQSGNSQESVTEQDSKDSTYSLSSTLTLSKADYEKHKVYACEVTHQGLSSPVTKSFNRGEC

SEQ ID NO: 12 - protein, 218 aa, Artificial Sequence
  anti-IL13-IGKC
DIVLTQSPASLAVSLGQRATISCRASESVDSYGQSYMHWYQQKAGQPPKLLIYLASNLESGVPARFSGSGSRTDFTLTIDPVQAEDAATYYCQQNAEDSRTFGGGTKLEIKRTVAAPSVFIFPPSDEQLKSGTASVVCLLNNFYPREAKVQWKVDNALQSGNSQESVTEQDSKDSTYSLSSTLTLSKADYEKHKVYACEVTHQGLSSPVTKSFNRGEC

SEQ ID NO: 13 - protein, 693 aa, Artificial Sequence
  anti-IL4-VH-huIGH-G11-huIGH-H1-<(G4S)3>-anti-IL13-VH-huIGHG1
QVQLQQSGPELVKPGASVKISCKASGYSFTSYWIHWIKQRPGQGLEWIGMIDPSDGETRLNQRFQGRATLTVDESTSTAYMQLRSPTSEDSAVYYCTRLKEYGNYDSFYFDVWGAGTLVTVSSASTKGPSVFPLAPSSKSTSGGTAALGCLVKDYFPEPVTVSWNSGALTSGVHTFPAVLQSSGLYSLSSVVTVPSSSLGTQTYICNVNHKPSNTKVDKKVEPKSCDKTHTGGGGSGGGGSGGGGSEVQLKESGPGLVAPGGSLSITCTVSGFSLTDSSINWVRQPPGKGLEWLGMIWGDGRIDYADALKSRLSISKDSSKSQVFLEMTSLRTDDTATYYCARDGYFPYAMDFWGQGTSVTVSSASTKGPSVFPLAPSSKSTSGGTAALGCLVKDYFPEPVTVSWNSGALTSGVHTFPAVLQSSGLYSLSSVVTVPSSSLGTQTYICNVNHKPSNTKVDKKVEPKSCDKTHTCPPCPAPELLGGPSVFLFPPKPKDTLMISRTPEVTCVVVDVSHEDPEVKFNWYVDGVEVHNAKTKPREEQYNSTYRVVSVLTVLHQDWLNGKEYKCKVSNKALPAPIEKTISKAKGQPREPQVYTLPPSRDELTKNQVSLTCLVKGFYPSDIAVEWESNGQPENNYKTTPPVLDSDGSFFLYSKLTVDKSRWQQGNVFSCSVMHEALHNHYTQKSLSLSPG

SEQ ID NO: 14 - protein, 446 aa, Artificial Sequence
  anti-IL4-VL-huIGKC-<G4S>-[PCS1]-<G4S>-anti-IL13-VL-huIGKC
DIQMTQSPASLSVSVGDTITLTCHASQNIDVWLSWFQQKPGNIPKLLIYKASNLHTGVPSRFSGSGSGTGFTLTISSLQPEDIATYYCQQAHSYPFTFGGGTKLEIKRTVAAPSVFIFPPSDEQLKSGTASVVCLLNNFYPREAKVQWKVDNALQSGNSQESVTEQDSKDSTYSLSSTLTLSKADYEKHKVYACEVTHQGLSSPVTKSFNRGECGGGGSRRKRGGGGSDIVLTQSPASLAVSLGQRATISCRASESVDSYGQSYMHWYQQKAGQPPKLLIYLASNLESGVPARFSGSGSRTDFTLTIDPVQAEDAATYYCQQNAEDSRTFGGGTKLEIKRTVAAPSVFIFPPSDEQLKSGTASVVCLLNNFYPREAKVQWKVDNALQSGNSQESVTEQDSKDSTYSLSSTLTLSKADYEKHKVYACEVTHQGLSSPVTKSFNRGEC

SEQ ID NO: 15 - protein, 455 aa, Artificial Sequence
  anti-IL4-VL-huIGKC-[PCS1]-<(G4S)3>-[PCS1]-anti-IL13-VL-huIGKC
DIQMTQSPASLSVSVGDTITLTCHASQNIDVWLSWFQQKPGNIPKLLIYKASNLHTGVPSRFSGSGSGTGFTLTISSLQPEDIATYYCQQAHSYPFTFGGGTKLEIKRTVAAPSVFIFPPSDEQLKSGTASVVCLLNNFYPREAKVQWKVDNALQSGNSQESVTEQDSKDSTYSLSSTLTLSKADYEKHKVYACEVTHQGLSSPVTKSFNRGECRRKRGGGGSGGGGSGGGGSRRKRDIVLTQSPASLAVSLGQRATISCRASESVDSYGQSYMHWYQQKAGQPPKLLIYLASNLESGVPARFSGSGSRTDFTLTIDPVQAEDAATYYCQQNAEDSRTFGGGTKLEIKRTVAAPSVFIFPPSDEQLKSGTASVVCLLNNFYPREAKVQWKVDNALQSGNSQESVTEQDSKDSTYSLSSTLTLSKADYEKHKVYACEVTHQGLSSPVTKSFNRGEC

SEQ ID NO: 16 - protein, 455 aa, Artificial Sequence
  anti-IL4-VL-huIGKC-[deltaPCS]-<(G4S)3>-[deltaPCS]-anti-IL13-VL-huIGKC
DIQMTQSPASLSVSVGDTITLTCHASQNIDVWLSWFQQKPGNIPKLLIYKASNLHTGVPSRFSGSGSGTGFTLTISSLQPEDIATYYCQQAHSYPFTFGGGTKLEIKRTVAAPSVFIFPPSDEQLKSGTASVVCLLNNFYPREAKVQWKVDNALQSGNSQESVTEQDSKDSTYSLSSTLTLSKADYEKHKVYACEVTHQGLSSPVTKSFNRGECRQQRGGGGSGGGGSGGGGSRQQRDIVLTQSPASLAVSLGQRATISCRASESVDSYGQSYMHWYQQKAGQPPKLLIYLASNLESGVPARFSGSGSRTDFTLTIDPVQAEDAATYYCQQNAEDSRTFGGGTKLEIKRTVAAPSVFIFPPSDEQLKSGTASVVCLLNNFYPREAKVQWKVDNALQSGNSQESVTEQDSKDSTYSLSSTLTLSKADYEKHKVYACEVTHQGLSSPVTKSFNRGEC

SEQ ID NO: 17 - protein, 455 aa, Artificial Sequence
  anti-IL4-VL-huIGKC-[PCS1]-<GS>-His(8)-<G4S>-[PCS1]-anti-IL13-VL-huIGKC
DIQMTQSPASLSVSVGDTITLTCHASQNIDVWLSWFQQKPGNIPKLLIYKASNLHTGVPSRFSGSGSGTGFTLTISSLQPEDIATYYCQQAHSYPFTFGGGTKLEIKRTVAAPSVFIFPPSDEQLKSGTASVVCLLNNFYPREAKVQWKVDNALQSGNSQESVTEQDSKDSTYSLSSTLTLSKADYEKHKVYACEVTHQGLSSPVTKSFNRGECRRKRGSHHHHHHHHGGGGSRRKRDIVLTQSPASLAVSLGQRATISCRASESVDSYGQSYMHWYQQKAGQPPKLLIYLASNLESGVPARFSGSGSRTDFTLTIDPVQAEDAATYYCQQNAEDSRTFGGGTKLEIKRTVAAPSVFIFPPSDEQLKSGTASVVCLLNNFYPREAKVQWKVDNALQSGNSQESVTEQDSKDSTYSLSSTLTLSKADYEKHKVYACEVTHQGLSSPVTKSFNRGEC

SEQ ID NO: 18 - protein, 455 aa, Artificial Sequence
  anti-IL4-VL-huIGKC-[deltaPCS]-<GS>-His(8)-<G4S>-[deltaPCS]-anti-IL13-VL-huIGKC
DIQMTQSPASLSVSVGDTITLTCHASQNIDVWLSWFQQKPGNIPKLLIYKASNLHTGVPSRFSGSGSGTGFTLTISSLQPEDIATYYCQQAHSYPFTFGGGTKLEIKRTVAAPSVFIFPPSDEQLKSGTASVVCLLNNFYPREAKVQWKVDNALQSGNSQESVTEQDSKDSTYSLSSTLTLSKADYEKHKVYACEVTHQGLSSPVTKSFNRGECRQQRGSHHHHHHHHGGGGSRQQRDIVLTQSPASLAVSLGQRATISCRASESVDSYGQSYMHWYQQKAGQPPKLLIYLASNLESGVPARFSGSGSRTDFTLTIDPVQAEDAATYYCQQNAEDSRTFGGGTKLEIKRTVAAPSVFIFPPSDEQLKSGTASVVCLLNNFYPREAKVQWKVDNALQSGNSQESVTEQDSKDSTYSLSSTLTLSKADYEKHKVYACEVTHQGLSSPVTKSFNRGEC

SEQ ID NO: 19 - protein, 457 aa, Artificial Sequence
  anti-IL4-VL-huIGKC-[PCS2]-<(G4S)3>-[PCS2]-anti-IL13-VL-huIGKC
DIQMTQSPASLSVSVGDTITLTCHASQNIDVWLSWFQQKPGNIPKLLIYKASNLHTGVPSRFSGSGSGTGFTLTISSLQPEDIATYYCQQAHSYPFTFGGGTKLEIKRTVAAPSVFIFPPSDEQLKSGTASVVCLLNNFYPREAKVQWKVDNALQSGNSQESVTEQDSKDSTYSLSSTLTLSKADYEKHKVYACEVTHQGLSSPVTKSFNRGECHRRRKRSVDEGGGGSHRRRKRSVDEDIVLTQSPASLAVSLGQRATISCRASESVDSYGQSYMHWYQQKAGQPPKLLIYLASNLESGVPARFSGSGSRTDFTLTIDPVQAEDAATYYCQQNAEDSRTFGGGTKLEIKRTVAAPSVFIFPPSDEQLKSGTASVVCLLNNFYPREAKVQWKVDNALQSGNSQESVTEQDSKDSTYSLSSTLTLSKADYEKHKVYACEVTHQGLSSPVTKSFNRGEC

SEQ ID NO: 20 - protein, 457 aa, Artificial Sequence
  anti-IL4-VL-huIGKC-[PCS3]-<(G4S)>-[PCS3]-anti-IL13-VL-huIGKC
DIQMTQSPASLSVSVGDTITLTCHASQNIDVWLSWFQQKPGNIPKLLIYKASNLHTGVPSRFSGSGSGTGFTLTISSLQPEDIATYYCQQAHSYPFTFGGGTKLEIKRTVAAPSVFIFPPSDEQLKSGTASVVCLLNNFYPREAKVQWKVDNALQSGNSQESVTEQDSKDSTYSLSSTLTLSKADYEKHKVYACEVTHQGLSSPVTKSFNRGECPMKKRRAGVPGGGGSPMKKRRAGVPDIVLTQSPASLAVSLGQRATISCRASESVDSYGQSYMHWYQQKAGQPPKLLIYLASNLESGVPARFSGSGSRTDFTLTIDPVQAEDAATYYCQQNAEDSRTFGGGTKLEIKRTVAAPSVFIFPPSDEQLKSGTASVVCLLNNFYPREAKVQWKVDNALQSGNSQESVTEQDSKDSTYSLSSTLTLSKADYEKHKVYACEVTHQGLSSPVTKSFNRGEC

SEQ ID NO: 21 - protein, 460 aa, Artificial Sequence
  anti-IL4-VL-huIGKC-[PCS1]-<G4S>-<(EAAAK)2>-<G4S>-[PCS1]-anti-IL13-VL-huIGKC
DIQMTQSPASLSVSVGDTITLTCHASQNIDVWLSWFQQKPGNIPKLLIYKASNLHTGVPSRFSGSGSGTGFTLTISSLQPEDIATYYCQQAHSYPFTFGGGTKLEIKRTVAAPSVFIFPPSDEQLKSGTASVVCLLNNFYPREAKVQWKVDNALQSGNSQESVTEQDSKDSTYSLSSTLTLSKADYEKHKVYACEVTHQGLSSPVTKSFNRGECRRKRGGGGSEAAAKEAAAKGGGGSRRKRDIVLTQSPASLAVSLGQRATISCRASESVDSYGQSYMHWYQQKAGQPPKLLIYLASNLESGVPARFSGSGSRTDFTLTIDPVQAEDAATYYCQQNAEDSRTFGGGTKLEIKRTVAAPSVFIFPPSDEQLKSGTASVVCLLNNFYPREAKVQWKVDNALQSGNSQESVTEQDSKDSTYSLSSTLTLSKADYEKHKVYACEVTHQGLSSPVTKSFNRGEC

SEQ ID NO: 22 - protein, 698 aa, Artificial Sequence
  anti-IL4-VH-huIGH-G11-huIGH-H1-<G4S>-<(EAAAK)2>-<G4S>-anti-IL13-VH-huIGHG1
QVQLQQSGPELVKPGASVKISCKASGYSFTSYWIHWIKQRPGQGLEWIGMIDPSDGETRLNQRFQGRATLTVDESTSTAYMQLRSPTSEDSAVYYCTRLKEYGNYDSFYFDVWGAGTLVTVSSASTKGPSVFPLAPSSKSTSGGTAALGCLVKDYFPEPVTVSWNSGALTSGVHTFPAVLQSSGLYSLSSVVTVPSSSLGTQTYICNVNHKPSNTKVDKKVEPKSCDKTHTGGGGSEAAAKEAAAKGGGGSEVQLKESGPGLVAPGGSLSITCTVSGFSLTDSSINWVRQPPGKGLEWLGMIWGDGRIDYADALKSRLSISKDSSKSQVFLEMTSLRTDDTATYYCARDGYFPYAMDFWGQGTSVTVSSASTKGPSVFPLAPSSKSTSGGTAALGCLVKDYFPEPVTVSWNSGALTSGVHTFPAVLQSSGLYSLSSVVTVPSSSLGTQTYICNVNHKPSNTKVDKKVEPKSCDKTHTCPPCPAPELLGGPSVFLFPPKPKDTLMISRTPEVTCVVVDVSHEDPEVKFNWYVDGVEVHNAKTKPREEQYNSTYRVVSVLTVLHQDWLNGKEYKCKVSNKALPAPIEKTISKAKGQPREPQVYTLPPSRDELTKNQVSLTCLVKGFYPSDIAVEWESNGQPENNYKTTPPVLDSDGSFFLYSKLTVDKSRWQQGNVFSCSVMHEALHNHYTQKSLSLSPG

SEQ ID NO: 23 - protein, 455 aa, Artificial Sequence
  anti-IL4-VL-huIGKC-[PCS1]-<(AP)7A>-[PCS1]-anti-IL13-VL-huIGKC
DIQMTQSPASLSVSVGDTITLTCHASQNIDVWLSWFQQKPGNIPKLLIYKASNLHTGVPSRFSGSGSGTGFTLTISSLQPEDIATYYCQQAHSYPFTFGGGTKLEIKRTVAAPSVFIFPPSDEQLKSGTASVVCLLNNFYPREAKVQWKVDNALQSGNSQESVTEQDSKDSTYSLSSTLTLSKADYEKHKVYACEVTHQGLSSPVTKSFNRGECRRKRAPAPAPAPAPAPAPARRKRDIVLTQSPASLAVSLGQRATISCRASESVDSYGQSYMHWYQQKAGQPPKLLIYLASNLESGVPARFSGSGSRTDFTLTIDPVQAEDAATYYCQQNAEDSRTFGGGTKLEIKRTVAAPSVFIFPPSDEQLKSGTASVVCLLNNFYPREAKVQWKVDNALQSGNSQESVTEQDSKDSTYSLSSTLTLSKADYEKHKVYACEVTHQGLSSPVTKSFNRGEC

SEQ ID NO: 24 - protein, 454 aa, Artificial Sequence
  anti-IL4-VL-huIGKC-[PCS1]-<GS>-<(KQGKQ)2>-<GS>-[PCS1]-anti-IL13-VL-huIGKC
DIQMTQSPASLSVSVGDTITLTCHASQNIDVWLSWFQQKPGNIPKLLIYKASNLHTGVPSRFSGSGSGTGFTLTISSLQPEDIATYYCQQAHSYPFTFGGGTKLEIKRTVAAPSVFIFPPSDEQLKSGTASVVCLLNNFYPREAKVQWKVDNALQSGNSQESVTEQDSKDSTYSLSSTLTLSKADYEKHKVYACEVTHQGLSSPVTKSFNRGECRRKRGSKQGKQKQGKQGSRRKRDIVLTQSPASLAVSLGQRATISCRASESVDSYGQSYMHWYQQKAGQPPKLLIYLASNLESGVPARFSGSGSRTDFTLTIDPVQAEDAATYYCQQNAEDSRTFGGGTKLEIKRTVAAPSVFIFPPSDEQLKSGTASVVCLLNNFYPREAKVQWKVDNALQSGNSQESVTEQDSKDSTYSLSSTLTLSKADYEKHKVYACEVTHQGLSSPVTKSFNRGEC

SEQ ID NO: 25 - protein, 686 aa, Artificial Sequence
  anti-IL4-VL-huIGKC-[PCS1]-<(G4S)3>-[PCS1]-anti-IL13-VL-huIGKC-<G4S>-Fc-huIgG1(hole-RF)
DIQMTQSPASLSVSVGDTITLTCHASQNIDVWLSWFQQKPGNIPKLLIYKASNLHTGVPSRFSGSGSGTGFTLTISSLQPEDIATYYCQQAHSYPFTFGGGTKLEIKRTVAAPSVFIFPPSDEQLKSGTASVVCLLNNFYPREAKVQWKVDNALQSGNSQESVTEQDSKDSTYSLSSTLTLSKADYEKHKVYACEVTHQGLSSPVTKSFNRGECRRKRGGGGSGGGGSGGGGSRRKRDIVLTQSPASLAVSLGQRATISCRASESVDSYGQSYMHWYQQKAGQPPKLLIYLASNLESGVPARFSGSGSRTDFTLTIDPVQAEDAATYYCQQNAEDSRTFGGGTKLEIKRTVAAPSVFIFPPSDEQLKSGTASVVCLLNNFYPREAKVQWKVDNALQSGNSQESVTEQDSKDSTYSLSSTLTLSKADYEKHKVYACEVTHQGLSSPVTKSFNRGECGGGGSDKTHTCPPCPAPELLGGPSVFLFPPKPKDTLMISRTPEVTCVVVDVSHEDPEVKFNWYVDGVEVHNAKTKPREEQYNSTYRVVSVLTVLHQDWLNGKEYKCKVSNKALPAPIEKTISKAKGQPREPQVCTLPPSRDELTKNQVSLSCAVKGFYPSDIAVEWESNGQPENNYKTTPPVLDSDGSFFLVSKLTVDKSRWQQGNVFSCSVMHEALHNRFTQKSLSLSPG

SEQ ID NO: 26 - protein, 693 aa, Artificial Sequence
  anti-IL4-VH-huIGH-G11-huIGH-H1-<(G4S)3>-anti-IL13-VH-huIGHG1(knob)
QVQLQQSGPELVKPGASVKISCKASGYSFTSYWIHWIKQRPGQGLEWIGMIDPSDGETRLNQRFQGRATLTVDESTSTAYMQLRSPTSEDSAVYYCTRLKEYGNYDSFYFDVWGAGTLVTVSSASTKGPSVFPLAPSSKSTSGGTAALGCLVKDYFPEPVTVSWNSGALTSGVHTFPAVLQSSGLYSLSSVVTVPSSSLGTQTYICNVNHKPSNTKVDKKVEPKSCDKTHTGGGGSGGGGSGGGGSEVQLKESGPGLVAPGGSLSITCTVSGFSLTDSSINWVRQPPGKGLEWLGMIWGDGRIDYADALKSRLSISKDSSKSQVFLEMTSLRTDDTATYYCARDGYFPYAMDFWGQGTSVTVSSASTKGPSVFPLAPSSKSTSGGTAALGCLVKDYFPEPVTVSWNSGALTSGVHTFPAVLQSSGLYSLSSVVTVPSSSLGTQTYICNVNHKPSNTKVDKKVEPKSCDKTHTCPPCPAPELLGGPSVFLFPPKPKDTLMISRTPEVTCVVVDVSHEDPEVKFNWYVDGVEVHNAKTKPREEQYNSTYRVVSVLTVLHQDWLNGKEYKCKVSNKALPAPIEKTISKAKGQPREPQVYTLPPCRDELTKNQVSLWCLVKGFYPSDIAVEWESNGQPENNYKTTPPVLDSDGSFFLYSKLTVDKSRWQQGNVFSCSVMHEALHNHYTQKSLSLSPG

SEQ ID NO: 27 - protein, 677 aa, Artificial Sequence
  anti-IL4-VL-huIGKC-<G4S>-[PCS1]-<G4S>-anti-IL13-VL-huIGKC-<G4S>-Fc-huIgG1(hole-RF)
DIQMTQSPASLSVSVGDTITLTCHASQNIDVWLSWFQQKPGNIPKLLIYKASNLHTGVPSRFSGSGSGTGFTLTISSLQPEDIATYYCQQAHSYPFTFGGGTKLEIKRTVAAPSVFIFPPSDEQLKSGTASVVCLLNNFYPREAKVQWKVDNALQSGNSQESVTEQDSKDSTYSLSSTLTLSKADYEKHKVYACEVTHQGLSSPVTKSFNRGECGGGGSRRKRGGGGSDIVLTQSPASLAVSLGQRATISCRASESVDSYGQSYMHWYQQKAGQPPKLLIYLASNLESGVPARFSGSGSRTDFTLTIDPVQAEDAATYYCQQNAEDSRTFGGGTKLEIKRTVAAPSVFIFPPSDEQLKSGTASVVCLLNNFYPREAKVQWKVDNALQSGNSQESVTEQDSKDSTYSLSSTLTLSKADYEKHKVYACEVTHQGLSSPVTKSFNRGECGGGGSDKTHTCPPCPAPELLGGPSVFLFPPKPKDTLMISRTPEVTCVVVDVSHEDPEVKFNWYVDGVEVHNAKTKPREEQYNSTYRVVSVLTVLHQDWLNGKEYKCKVSNKALPAPIEKTISKAKGQPREPQVCTLPPSRDELTKNQVSLSCAVKGFYPSDIAVEWESNGQPENNYKTTPPVLDSDGSFFLVSKLTVDKSRWQQGNVFSCSVMHEALHNRFTQKSLSLSPG

SEQ ID NO: 28 - protein, 686 aa, Artificial Sequence
  anti-IL4-VL-huIGKC-[deltaPCS]-<(G4S)3>-[deltaPCS]-anti-IL13-VL-huIGKC-<G4S>-Fc-huIgG1(hole-RF)
DIQMTQSPASLSVSVGDTITLTCHASQNIDVWLSWFQQKPGNIPKLLIYKASNLHTGVPSRFSGSGSGTGFTLTISSLQPEDIATYYCQQAHSYPFTFGGGTKLEIKRTVAAPSVFIFPPSDEQLKSGTASVVCLLNNFYPREAKVQWKVDNALQSGNSQESVTEQDSKDSTYSLSSTLTLSKADYEKHKVYACEVTHQGLSSPVTKSFNRGECRQQRGGGGSGGGGSGGGGSRQQRDIVLTQSPASLAVSLGQRATISCRASESVDSYGQSYMHWYQQKAGQPPKLLIYLASNLESGVPARFSGSGSRTDFTLTIDPVQAEDAATYYCQQNAEDSRTFGGGTKLEIKRTVAAPSVFIFPPSDEQLKSGTASVVCLLNNFYPREAKVQWKVDNALQSGNSQESVTEQDSKDSTYSLSSTLTLSKADYEKHKVYACEVTHQGLSSPVTKSFNRGECGGGGSDKTHTCPPCPAPELLGGPSVFLFPPKPKDTLMISRTPEVTCVVVDVSHEDPEVKFNWYVDGVEVHNAKTKPREEQYNSTYRVVSVLTVLHQDWLNGKEYKCKVSNKALPAPIEKTISKAKGQPREPQVCTLPPSRDELTKNQVSLSCAVKGFYPSDIAVEWESNGQPENNYKTTPPVLDSDGSFFLVSKLTVDKSRWQQGNVFSCSVMHEALHNRFTQKSLSLSPG

SEQ ID NO: 29 - protein, 686 aa, Artificial Sequence
  anti-IL4-VL-huIGKC-[PCS1]-<GS>-His(8)-<G4S>-[PCS1]-anti-IL13-VL-huIGKC-<G4S>-Fc-huIgG1(hole-RF)
DIQMTQSPASLSVSVGDTITLTCHASQNIDVWLSWFQQKPGNIPKLLIYKASNLHTGVPSRFSGSGSGTGFTLTISSLQPEDIATYYCQQAHSYPFTFGGGTKLEIKRTVAAPSVFIFPPSDEQLKSGTASVVCLLNNFYPREAKVQWKVDNALQSGNSQESVTEQDSKDSTYSLSSTLTLSKADYEKHKVYACEVTHQGLSSPVTKSFNRGECRRKRGSHHHHHHHHGGGGSRRKRDIVLTQSPASLAVSLGQRATISCRASESVDSYGQSYMHWYQQKAGQPPKLLIYLASNLESGVPARFSGSGSRTDFTLTIDPVQAEDAATYYCQQNAEDSRTFGGGTKLEIKRTVAAPSVFIFPPSDEQLKSGTASVVCLLNNFYPREAKVQWKVDNALQSGNSQESVTEQDSKDSTYSLSSTLTLSKADYEKHKVYACEVTHQGLSSPVTKSFNRGECGGGGSDKTHTCPPCPAPELLGGPSVFLFPPKPKDTLMISRTPEVTCVVVDVSHEDPEVKFNWYVDGVEVHNAKTKPREEQYNSTYRVVSVLTVLHQDWLNGKEYKCKVSNKALPAPIEKTISKAKGQPREPQVCTLPPSRDELTKNQVSLSCAVKGFYPSDIAVEWESNGQPENNYKTTPPVLDSDGSFFLVSKLTVDKSRWQQGNVFSCSVMHEALHNRFTQKSLSLSPG

SEQ ID NO: 30 - protein, 686 aa, Artificial Sequence
  anti-IL4-VL-huIGKC-[deltaPCS]-<GS>-His(8)-<G4S>-[deltaPCS]-anti-IL13-VL-huIGKC-<G4S>-Fc-huIgG1(hole-RF)
DIQMTQSPASLSVSVGDTITLTCHASQNIDVWLSWFQQKPGNIPKLLIYKASNLHTGVPSRFSGSGSGTGFTLTISSLQPEDIATYYCQQAHSYPFTFGGGTKLEIKRTVAAPSVFIFPPSDEQLKSGTASVVCLLNNFYPREAKVQWKVDNALQSGNSQESVTEQDSKDSTYSLSSTLTLSKADYEKHKVYACEVTHQGLSSPVTKSFNRGECRQQRGSHHHHHHHHGGGGSRQQRDIVLTQSPASLAVSLGQRATISCRASESVDSYGQSYMHWYQQKAGQPPKLLIYLASNLESGVPARFSGSGSRTDFTLTIDPVQAEDAATYYCQQNAEDSRTFGGGTKLEIKRTVAAPSVFIFPPSDEQLKSGTASVVCLLNNFYPREAKVQWKVDNALQSGNSQESVTEQDSKDSTYSLSSTLTLSKADYEKHKVYACEVTHQGLSSPVTKSFNRGECGGGGSDKTHTCPPCPAPELLGGPSVFLFPPKPKDTLMISRTPEVTCVVVDVSHEDPEVKFNWYVDGVEVHNAKTKPREEQYNSTYRVVSVLTVLHQDWLNGKEYKCKVSNKALPAPIEKTISKAKGQPREPQVCTLPPSRDELTKNQVSLSCAVKGFYPSDIAVEWESNGQPENNYKTTPPVLDSDGSFFLVSKLTVDKSRWQQGNVFSCSVMHEALHNRFTQKSLSLSPG

SEQ ID NO: 31 - protein, 688 aa, Artificial Sequence
  anti-IL4-VL-huIGKC-[PCS2]-<(G4S)3>-[PCS2]-anti-IL13-VL-huIGKC-<G4S>-Fc-huIgG1(hole-RF)
DIQMTQSPASLSVSVGDTITLTCHASQNIDVWLSWFQQKPGNIPKLLIYKASNLHTGVPSRFSGSGSGTGFTLTISSLQPEDIATYYCQQAHSYPFTFGGGTKLEIKRTVAAPSVFIFPPSDEQLKSGTASVVCLLNNFYPREAKVQWKVDNALQSGNSQESVTEQDSKDSTYSLSSTLTLSKADYEKHKVYACEVTHQGLSSPVTKSFNRGECHRRRKRSVDEGGGGSHRRRKRSVDEDIVLTQSPASLAVSLGQRATISCRASESVDSYGQSYMHWYQQKAGQPPKLLIYLASNLESGVPARFSGSGSRTDFTLTIDPVQAEDAATYYCQQNAEDSRTFGGGTKLEIKRTVAAPSVFIFPPSDEQLKSGTASVVCLLNNFYPREAKVQWKVDNALQSGNSQESVTEQDSKDSTYSLSSTLTLSKADYEKHKVYACEVTHQGLSSPVTKSFNRGECGGGGSDKTHTCPPCPAPELLGGPSVFLFPPKPKDTLMISRTPEVTCVVVDVSHEDPEVKFNWYVDGVEVHNAKTKPREEQYNSTYRVVSVLTVLHQDWLNGKEYKCKVSNKALPAPIEKTISKAKGQPREPQVCTLPPSRDELTKNQVSLSCAVKGFYPSDIAVEWESNGQPENNYKTTPPVLDSDGSFFLVSKLTVDKSRWQQGNVFSCSVMHEALHNRFTQKSLSLSPG

SEQ ID NO: 32 - protein, 688 aa, Artificial Sequence
  anti-IL4-VL-huIGKC-[PCS3]-<(G4S)3>-[PCS3]-anti-IL13-VL-huIGKC-<G4S>-Fc-huIgG1(hole-RF)
DIQMTQSPASLSVSVGDTITLTCHASQNIDVWLSWFQQKPGNIPKLLIYKASNLHTGVPSRFSGSGSGTGFTLTISSLQPEDIATYYCQQAHSYPFTFGGGTKLEIKRTVAAPSVFIFPPSDEQLKSGTASVVCLLNNFYPREAKVQWKVDNALQSGNSQESVTEQDSKDSTYSLSSTLTLSKADYEKHKVYACEVTHQGLSSPVTKSFNRGECPMKKRRAGVPGGGGSPMKKRRAGVPDIVLTQSPASLAVSLGQRATISCRASESVDSYGQSYMHWYQQKAGQPPKLLIYLASNLESGVPARFSGSGSRTDFTLTIDPVQAEDAATYYCQQNAEDSRTFGGGTKLEIKRTVAAPSVFIFPPSDEQLKSGTASVVCLLNNFYPREAKVQWKVDNALQSGNSQESVTEQDSKDSTYSLSSTLTLSKADYEKHKVYACEVTHQGLSSPVTKSFNRGECGGGGSDKTHTCPPCPAPELLGGPSVFLFPPKPKDTLMISRTPEVTCVVVDVSHEDPEVKFNWYVDGVEVHNAKTKPREEQYNSTYRVVSVLTVLHQDWLNGKEYKCKVSNKALPAPIEKTISKAKGQPREPQVCTLPPSRDELTKNQVSLSCAVKGFYPSDIAVEWESNGQPENNYKTTPPVLDSDGSFFLVSKLTVDKSRWQQGNVFSCSVMHEALHNRFTQKSLSLSPG

SEQ ID NO: 33 - protein, 691 aa, Artificial Sequence
  anti-IL4-VL-huIGKC-[PCS1]-<G4S>-<(EAAAK)2>-<G4S>-[PCS1]-anti-IL13-VL-huIGKC-<G4S>-Fc-huIgG1(hole-RF)
DIQMTQSPASLSVSVGDTITLTCHASQNIDVWLSWFQQKPGNIPKLLIYKASNLHTGVPSRFSGSGSGTGFTLTISSLQPEDIATYYCQQAHSYPFTFGGGTKLEIKRTVAAPSVFIFPPSDEQLKSGTASVVCLLNNFYPREAKVQWKVDNALQSGNSQESVTEQDSKDSTYSLSSTLTLSKADYEKHKVYACEVTHQGLSSPVTKSFNRGECRRKRGGGGSEAAAKEAAAKGGGGSRRKRDIVLTQSPASLAVSLGQRATISCRASESVDSYGQSYMHWYQQKAGQPPKLLIYLASNLESGVPARFSGSGSRTDFTLTIDPVQAEDAATYYCQQNAEDSRTFGGGTKLEIKRTVAAPSVFIFPPSDEQLKSGTASVVCLLNNFYPREAKVQWKVDNALQSGNSQESVTEQDSKDSTYSLSSTLTLSKADYEKHKVYACEVTHQGLSSPVTKSFNRGECGGGGSDKTHTCPPCPAPELLGGPSVFLFPPKPKDTLMISRTPEVTCVVVDVSHEDPEVKFNWYVDGVEVHNAKTKPREEQYNSTYRVVSVLTVLHQDWLNGKEYKCKVSNKALPAPIEKTISKAKGQPREPQVCTLPPSRDELTKNQVSLSCAVKGFYPSDIAVEWESNGQPENNYKTTPPVLDSDGSFFLVSKLTVDKSRWQQGNVFSCSVMHEALHNRFTQKSLSLSPG

SEQ ID NO: 34 - protein, 698 aa, Artificial Sequence
  anti-IL4-VH-huIGH-G11-huIGH-H1-<G4S>-<(EAAAK)2>-<G4S>-anti-IL13-VH-huIGHG1(knob)
QVQLQQSGPELVKPGASVKISCKASGYSFTSYWIHWIKQRPGQGLEWIGMIDPSDGETRLNQRFQGRATLTVDESTSTAYMQLRSPTSEDSAVYYCTRLKEYGNYDSFYFDVWGAGTLVTVSSASTKGPSVFPLAPSSKSTSGGTAALGCLVKDYFPEPVTVSWNSGALTSGVHTFPAVLQSSGLYSLSSVVTVPSSSLGTQTYICNVNHKPSNTKVDKKVEPKSCDKTHTGGGGSEAAAKEAAAKGGGGSEVQLKESGPGLVAPGGSLSITCTVSGFSLTDSSINWVRQPPGKGLEWLGMIWGDGRIDYADALKSRLSISKDSSKSQVFLEMTSLRTDDTATYYCARDGYFPYAMDFWGQGTSVTVSSASTKGPSVFPLAPSSKSTSGGTAALGCLVKDYFPEPVTVSWNSGALTSGVHTFPAVLQSSGLYSLSSVVTVPSSSLGTQTYICNVNHKPSNTKVDKKVEPKSCDKTHTCPPCPAPELLGGPSVFLFPPKPKDTLMISRTPEVTCVVVDVSHEDPEVKFNWYVDGVEVHNAKTKPREEQYNSTYRVVSVLTVLHQDWLNGKEYKCKVSNKALPAPIEKTISKAKGQPREPQVYTLPPCRDELTKNQVSLWCLVKGFYPSDIAVEWESNGQPENNYKTTPPVLDSDGSFFLYSKLTVDKSRWQQGNVFSCSVMHEALHNHYTQKSLSLSPG

SEQ ID NO: 35 - protein, 686 aa, Artificial Sequence
  anti-IL4-VL-huIGKC-[PCS1]-<(AP)7A>-[PCS1]-anti-IL13-VL-huIGKC-<G4S>-Fc-huIgG1(hole-RF)
DIQMTQSPASLSVSVGDTITLTCHASQNIDVWLSWFQQKPGNIPKLLIYKASNLHTGVPSRFSGSGSGTGFTLTISSLQPEDIATYYCQQAHSYPFTFGGGTKLEIKRTVAAPSVFIFPPSDEQLKSGTASVVCLLNNFYPREAKVQWKVDNALQSGNSQESVTEQDSKDSTYSLSSTLTLSKADYEKHKVYACEVTHQGLSSPVTKSFNRGECRRKRAPAPAPAPAPAPAPARRKRDIVLTQSPASLAVSLGQRATISCRASESVDSYGQSYMHWYQQKAGQPPKLLIYLASNLESGVPARFSGSGSRTDFTLTIDPVQAEDAATYYCQQNAEDSRTFGGGTKLEIKRTVAAPSVFIFPPSDEQLKSGTASVVCLLNNFYPREAKVQWKVDNALQSGNSQESVTEQDSKDSTYSLSSTLTLSKADYEKHKVYACEVTHQGLSSPVTKSFNRGECGGGGSDKTHTCPPCPAPELLGGPSVFLFPPKPKDTLMISRTPEVTCVVVDVSHEDPEVKFNWYVDGVEVHNAKTKPREEQYNSTYRVVSVLTVLHQDWLNGKEYKCKVSNKALPAPIEKTISKAKGQPREPQVCTLPPSRDELTKNQVSLSCAVKGFYPSDIAVEWESNGQPENNYKTTPPVLDSDGSFFLVSKLTVDKSRWQQGNVFSCSVMHEALHNRFTQKSLSLSPG

SEQ ID NO: 36 - protein, 685 aa, Artificial Sequence
  anti-IL4-VL-huIGKC-[PCS1]-<GS>-<(KQGKQ)2>-<GS>-[PCS1]-anti-IL13-VL-huIGKC-<G4S>-Fc-huIgG1(hole-RF)
DIQMTQSPASLSVSVGDTITLTCHASQNIDVWLSWFQQKPGNIPKLLIYKASNLHTGVPSRFSGSGSGTGFTLTISSLQPEDIATYYCQQAHSYPFTFGGGTKLEIKRTVAAPSVFIFPPSDEQLKSGTASVVCLLNNFYPREAKVQWKVDNALQSGNSQESVTEQDSKDSTYSLSSTLTLSKADYEKHKVYACEVTHQGLSSPVTKSFNRGECRRKRGSKQGKQKQGKQGSRRKRDIVLTQSPASLAVSLGQRATISCRASESVDSYGQSYMHWYQQKAGQPPKLLIYLASNLESGVPARFSGSGSRTDFTLTIDPVQAEDAATYYCQQNAEDSRTFGGGTKLEIKRTVAAPSVFIFPPSDEQLKSGTASVVCLLNNFYPREAKVQWKVDNALQSGNSQESVTEQDSKDSTYSLSSTLTLSKADYEKHKVYACEVTHQGLSSPVTKSFNRGECGGGGSDKTHTCPPCPAPELLGGPSVFLFPPKPKDTLMISRTPEVTCVVVDVSHEDPEVKFNWYVDGVEVHNAKTKPREEQYNSTYRVVSVLTVLHQDWLNGKEYKCKVSNKALPAPIEKTISKAKGQPREPQVCTLPPSRDELTKNQVSLSCAVKGFYPSDIAVEWESNGQPENNYKTTPPVLDSDGSFFLVSKLTVDKSRWQQGNVFSCSVMHEALHNRFTQKSLSLSPG

SEQ ID NO: 37 - protein, 768 aa, Homo sapiens
QKVFTNTWAVRIPGGPAVANSVARKHGFLNLGQIFGDYYHFWHRGVTKRSLSPHRPRHSRLQREPQVQWLEQQVAKRRTKRDVYQEPTDPKFPQQWYLSGVTQRDLNVKAAWAQGYTGHGIVVSILDDGIEKNHPDLAGNYDPGASFDVNDQDPDPQPRYTQMNDNRHGTRCAGEVAAVANNGVCGVGVAYNARIGGVRMLDGEVTDAVEARSLGLNPNHIHIYSASWGPEDDGKTVDGPARLAEEAFFRGVSQGRGGLGSIFVWASGNGGREHDSCNCDGYTNSIYTLSISSATQFGNVPWYSEACSSTLATTYSSGNQNEKQIVTTDLRQKCTESHTGTSASAPLAAGIIALTLEANKNLTWRDMQHLVVQTSKPAHLNANDWATNGVGRKVSHSYGYGLLDAGAMVALAQNWTTVAPQRKCIIDILTEPKDIGKRLEVRKTVTACLGEPNHITRLEHAQARLTLSYNRRGDLAIHLVSPMGTRSTLLAARPHDYSADGFNDWAFMTTHSWDEDPSGEWVLEIENTSEANNYGTLTKFTLVLYGTAPEGLPVPPESSGCKTLTSSQACVVCEEGFSLHQKSCVQHCPPGFAPQVLDTHYSTENDVETIRASVCAPCHASCATCQGPALTDCLSCPSHASLDPVEQTCSRQSQSSRESPPQQQPPRLPPEVEAGQRLRAGLLPSHLPEVVAGLSCAFIVLVFVTVFLVLQLRSGFSFRGVKVYTMDRGLISYKGLPPEAWQEECPSDSEEDEGRGERTAFIKDQSAL

SEQ ID NO: 38 - protein, 775 aa, Artificial Sequence
  Propeptide Furin-mature Furin-<GAA>-KDEL signal peptide
QKVFTNTWAVRIPGGPAVANSVARKHGFLNLGQIFGDYYHFWHRGVTKRSLSPHRPRHSRLQREPQVQWLEQQVAKRRTKRDVYQEPTDPKFPQQWYLSGVTQRDLNVKAAWAQGYTGHGIVVSILDDGIEKNHPDLAGNYDPGASFDVNDQDPDPQPRYTQMNDNRHGTRCAGEVAAVANNGVCGVGVAYNARIGGVRMLDGEVTDAVEARSLGLNPNHIHIYSASWGPEDDGKTVDGPARLAEEAFFRGVSQGRGGLGSIFVWASGNGGREHDSCNCDGYTNSIYTLSISSATQFGNVPWYSEACSSTLATTYSSGNQNEKQIVTTDLRQKCTESHTGTSASAPLAAGIIALTLEANKNLTWRDMQHLVVQTSKPAHLNANDWATNGVGRKVSHSYGYGLLDAGAMVALAQNWTTVAPQRKCIIDILTEPKDIGKRLEVRKTVTACLGEPNHITRLEHAQARLTLSYNRRGDLAIHLVSPMGTRSTLLAARPHDYSADGFNDWAFMTTHSWDEDPSGEWVLEIENTSEANNYGTLTKFTLVLYGTAPEGLPVPPESSGCKTLTSSQACVVCEEGFSLHQKSCVQHCPPGFAPQVLDTHYSTENDVETIRASVCAPCHASCATCQGPALTDCLSCPSHASLDPVEQTCSRQSQSSRESPPQQQPPRLPPEVEAGQRLRAGLLPSHLPEVVAGLSCAFIVLVFVTVFLVLQLRSGFSFRGVKVYTMDRGLISYKGLPPEAWQEECPSDSEEDEGRGERTAFIKDQSALGAAKDEL

SEQ ID NO: 39 - protein, 1828 aa, Homo sapiens
RVYTNHWAVKIAGGFPEANRIASKYGFINIGQIGALKDYYHFYHSRTIKRSVISSRGTHSFISMEPKVEWIQQQVVKKRTKRDYDFSRAQSTYFNDPKWPSMWYMHCSDNTHPCQSDMNIEGAWKRGYTGKNIVVTILDDGIERTHPDLMQNYDALASCDVNGNDLDPMPRYDASNENKHGTRCAGEVAAAANNSHCTVGIAFNAKIGGVRMLDGDVTDMVEAKSVSFNPQHVHIYSASWGPDDDGKTVDGPAPLTRQAFENGVRMGRRGLGSVFVWASGNGGRSKDHCSCDGYTNSIYTISISSTAESGKKPWYLEECSSTLATTYSSGESYDKKIITTDLRQRCTDNHTGTSASAPMAAGIIALALEANPFLTWRDVQHVIVRTSRAGHLNANDWKTNAAGFKVSHLYGFGLMDAEAMVMEAEKWTTVPRQHVCVESTDRQIKTIRPNSAVRSIYKASGCSDNPNRHVNYLEHVVVRITITHPRRGDLAIYLTSPSGTRSQLLANRLFDHSMEGFKNWEFMTIHCWGERAAGDWVLEVYDTPSQLRNFKTPGKLKEWSLVLYGTSVQPYSPTNEFPKVERFRYSRVEDPTDDYGTEDYAGPCDPECSEVGCDGPGPDHCNDCLHYYYKLKNNTRICVSSCPPGHYHADKKRCRKCAPNCESCFGSHGDQCMSCKYGYFLNEETNSCVTHCPDGSYQDTKKNLCRKCSENCKTCTEFHNCTECRDGLSLQGSRCSVSCEDGRYFNGQDCQPCHRFCATCAGAGADGCINCTEGYFMEDGRCVQSCSISYYFDHSSENGYKSCKKCDISCLTCNGPGFKNCTSCPSGYLLDLGMCQMGAICKDGEYVDEHGHCQTCEASCAKCQGPTQEDCTTCPMTRIFDDGRCVSNCPSWKFEFENQCHPCHHTCQRCQGSGPTHCTSCGADNYGREHFLYQGECGDSCPEGHYATEGNTCLPCPDNCELCHSVHVCTRCMKGYFIAPTNHTCQKLECGQGEVQDPDYEECVPCEEGCLGCSLDDPGTCTSCAMGYYRFDHHCYKTCPEKTYSEEVECKACDSNCGSCDQNGCYWCEEGFFLLGGSCVRKCGPGFYGDQEMGECESCHRACETCTGPGHDECSSCQEGLQLLRGMCVHATKTQEEGKFWNDILRKLQPCHSSCKTCNGSATLCTSCPKGAYLLAQACVSSCPQGTWPSVRSGSCENCTEACAICSGADLCKKCQMQPGHPLFLHEGRCYSKCPEGSYAEDGICERCSSPCRTCEGNATNCHSCEGGHVLHHGVCQENCPERHVAVKGVCKHCPEMCQDCIHEKTCKECTPEFFLHDDMCHQSCPRGFYADSRHCVPCHKDCLECSGPKADDCELCLESSWVLYDGLCLEECPAGTYYEKETKECRDCHKSCLTCSSSGTCTTCQKGLIMNPRGSCMANEKCSPSEYWDEDAPGCKPCHVKCFHCMGPAEDQCQTCPMNSLLLNTTCVKDCPEGYYADEDSNRCAHCHSSCRTCEGRHSRQCHSCRPGWFQLGKECLLQCREGYYADNSTGRCERCNRSCKGCQGPRPTDCLSCDRFFFLLRSKGECHRSCPDHYYVEQSTQTCERCHPTCDQCKGKGALNCLSCVWSYHLMGGICTSDCLVGEYRVGEGEKFNCEKCHESCMECKGPGAKNCTLCPANLVLHMDDSHCLHCCNTSDPPSAQECCDCQDTTDECILRTSKVRPATEHFKTALFITSSMMLVLLLGAAVVVWKKSRGRVQPAAKAGYEKLADPNKSYSSYKSSYRESTSFEEDQVIEYRDRDYDEDDDDDIVYMGQDGTVYRKFKYGLLDDDDIDELEYDDESYSYYQ

SEQ ID NO: 40 - protein, 748 aa, Homo sapiens
LAGTGGPDGQGTGGPSWAVHLESLEGDGEEETLEQQADALAQAAGLVNAGRIGELQGHYLFVQPAGHRPALEVEAIRQQVEAVLAGHEAVRWHSEQRLLRRAKRSVHFNDPKYPQQWHLNNRRSPGRDINVTGVWERNVTGRGVTVVVVDDGVEHTIQDIAPNYSPEGSYDLNSNDPDPMPHPDVENGNHHGTRCAGEIAAVPNNSFCAVGVAYGSRIAGIRVLDGPLTDSMEAVAFNKHYQINDIYSCSWGPDDDGKTVDGPHQLGKAALQHGVIAGRQGFGSIFVVASGNGGQHNDNCNYDGYANSIYTVTIGAVDEEGRMPFYAEECASMLAVTFSGGDKMLRSIVTTDWDLQKGTGCTEGHTGTSAAAPLAAGMIALMLQVRPCLTWRDVQHIIVFTATRYEDRRAEWVTNEAGFSHSHQHGFGLLNAWRLVNAAKIWTSVPYLASYVSPVLKENKAIPQSPRSLEVLWNVSRMDLEMSGLKTLEHVAVTVSITHPRRGSLELKLFCPSGMMSLIGAPRSMDSDPNGFNDWTFSTVRCWGERARGTYRLVIRDVGDESFQVGILRQWQLTLYGSVWSAVDIRDRQRLLESAMSGKYLHDDFALPCPPGLKIPEEDGYTITPNTLKTLVLVGCFTVFWTVYYMLEVYLSQRNVASNQVCRSGPCHWPHRSRKAKEEGTELESVPLCSSKDPDEVETESRGPPTTSDLLAPDLLEQGDWSLSQNKSALDCPHQHLDVPHGKEEQIC

SEQ ID NO: 41 - protein, 906 aa, Homo sapiens
PPPRPVYTNHWAVQVLGGPAEADRVAAAHGYLNLGQIGNLEDYYHFYHSKTFKRSTLSSRGPHTFLRMDPQVKWLQQQEVKRRVKRQVRSDPQALYFNDPIWSNMWYLHCGDKNSRCRSEMNVQAAWKRGYTGKNVVVTILDDGIERNHPDLAPNYDSYASYDVNGNDYDPSPRYDASNENKHGTRCAGEVAASANNSYCIVGIAYNAKIGGIRMLDGDVTDVVEAKSLGIRPNYIDIYSASWGPDDDGKTVDGPGRLAKQAFEYGIKKGRQGLGSIFVWASGNGGREGDYCSCDGYTNSIYTISVSSATENGYKPWYLEECASTLATTYSSGAFYERKIVTTDLRQRCTDGHTGTSVSAPMVAGIIALALEANSQLTWRDVQHLLVKTSRPAHLKASDWKVNGAGHKVSHFYGFGLVDAEALVVEAKKWTAVPSQHMCVAASDKRPRSIPLVQVLRTTALTSACAEHSDQRVVYLEHVVVRTSISHPRRGDLQIYLVSPSGTKSQLLAKRLLDLSNEGFTNWEFMTVHCWGEKAEGQWTLEIQDLPSQVRNPEKQGKLKEWSLILYGTAEHPYHTFSAHQSRSRMLELSAPELEPPKAALSPSQVEVPEDEEDYTAQSTPGSANILQTSVCHPECGDKGCDGPNADQCLNCVHFSLGSVKTSRKCVSVCPLGYFGDTAARRCRRCHKGCETCSSRAATQCLSCRRGFYHHQEMNTCVTLCPAGFYADESQKNCLKCHPSCKKCVDEPEKCTVCKEGFSLARGSCIPDCEPGTYFDSELIRCGECHHTCGTCVGPGREECIHCAKNFHFHDWKCVPACGEGFYPEEMPGLPHKVCRRCDENCLSCAGSSRNCSRCKTGFTQLGTSCITNHTCSNADETFCEMVKSNRLCERKLFIQFCCRTCLLAG

SEQ ID NO: 42 - protein, 10 aa, Artificial Sequence
  PCS General Formula
  misc_feature (4)..(5): Xaa can be any naturally occurring amino acid
HRRXXRSVDE

SEQ ID NO: 43 - protein, 10 aa, Artificial Sequence
  PCS2
HRRRKRSVDE

SEQ ID NO: 44 - protein, 10 aa, Artificial Sequence
  PCS2a
HRRQQRSVDE

SEQ ID NO: 45 - protein, 15 aa, Artificial Sequence
  Linker
GSHHHHHHHHGGGGS

SEQ ID NO: 46 - protein, 20 aa, Artificial Sequence
  Linker
GGGGSEAAAKEAAAKGGGGS

SEQ ID NO: 47 - protein, 15 aa, Artificial Sequence
  Linker
APAPAPAPAPAPAPA

SEQ ID NO: 48 - protein, 14 aa, Artificial Sequence
  Linker
GSKQGKQKQGKQGS

SEQ ID NO: 49 - protein, 4 aa, Artificial Sequence
  PCS1
RRKR

SEQ ID NO: 50 - protein, 10 aa, Artificial Sequence
  PCS3
PMKKRRAGVP

SEQ ID NO: 51 - protein, 5 aa, Artificial Sequence
  Linker
  REPEAT (1)..(5)
GGGGS

SEQ ID NO: 52 - protein, 5 aa, Artificial Sequence
  Linker
  REPEAT (1)..(5)
EAAAK

SEQ ID NO: 53 - protein, 3 aa, Artificial Sequence
  Linker
  REPEAT (1)..(2)
APA

SEQ ID NO: 54 - protein, 5 aa, Artificial Sequence
  Linker
  REPEAT (1)..(5)
KQGKQ

SEQ ID NO: 55 - protein, 15 aa, Artificial Sequence
  Linker
GGGGSGGGGSGGGGS

SEQ ID NO: 56 - protein, 341 aa, Artificial Sequence
  anti-OX40-VL-<(G4S)2>-anti-PD1-VL-<(G4S)2>-huIGKC
DIQMTQSPSSLSASVGDRVTITCRASQDISNYLNWYQQKPGKAPKLLIYYTSRLRSGVPSRFSGSGSGTDFTLTISSLQPEDFATYYCQQGHTLPPTFGQGTKVEIKGGGGSGGGGSEIVLTQSPATLSLSPGERATLSCRASQSVSSYLAWYQQKPGQAPRLLIYDASNRATGIPARFSGSGSGTDFTLTISSLEPEDFAVYYCQQSSNWPRTFGQGTKVEIKGGGGSGGGGSRTVAAPSVFIFPPSDEQLKSGTASVVCLLNNFYPREAKVQWKVDNALQSGNSQESVTEQDSKDSTYSLSSTLTLSKADYEKHKVYACEVTHQGLSSPVTKSFNRGEC

SEQ ID NO: 57 - protein, 559 aa, Artificial Sequence
  anti-PD1-VH-anti-OX40-VH-huIGHG1(LALA-knob)
QVQLVESGGGVVQPGRSLRLDCKASGITFSNSGMHWVRQAPGKGLEWVAVIWYDGSKRYYADSVKGRFTISRDNSKNTLFLQMNSLRAEDTAVYYCATNDDYWGQGTLVTVSSEVQLVQSGAEVKKPGASVKVSCKASGYTFTDSYMSWVRQAPGQGLEWIGDMYPDNGDSSYNQKFRERVTITRDTSTSTAYLELSSLRSEDTAVYYCVLAPRWYFSVWGQGTLVTVSSASTKGPSVFPLAPSSKSTSGGTAALGCLVKDYFPEPVTVSWNSGALTSGVHTFPAVLQSSGLYSLSSVVTVPSSSLGTQTYICNVNHKPSNTKVDKKVEPKSCDKTHTCPPCPAPEAAGGPSVFLFPPKPKDTLMISRTPEVTCVVVDVSHEDPEVKFNWYVDGVEVHNAKTKPREEQYNSTYRVVSVLTVLHQDWLNGKEYKCKVSNKALPAPIEKTISKAKGQPREPQVYTLPPCRDELTKNQVSLWCLVKGFYPSDIAVEWESNGQPENNYKTTPPVLDSDGSFFLYSKLTVDKSRWQQGNVFSCSVMHEALHNHYTQKSLSLSPG

SEQ ID NO: 58 - protein, 214 aa, Artificial Sequence
  anti-GITR-VL-huIGKC
AIQLTQSPSSLSASVGDRVTITCRASQGISSALAWYQQKPGKAPKLLIYDASSLESGVPSRFSGSGSGTDFTLTISSLQPEDFATYYCQQFNSYPYTFGQGTKLEIKRTVAAPSVFIFPPSDEQLKSGTASVVCLLNNFYPREAKVQWKVDNALQSGNSQESVTEQDSKDSTYSLSSTLTLSKADYEKHKVYACEVTHQGLSSPVTKSFNRGEC

SEQ ID NO: 59 - protein, 453 aa, Artificial Sequence
  anti-GITR-VH-huIGHG1(LALA-hole-RF)
QVQLVESGGGVVQPGRSLRLSCAASGFTFSSYGMHWVRQAPGKGLEWVAVIWYEGSNKYYADSVKGRFTISRDNSKNTLYLQMNSLRAEDTAVYYCARGGSMVRGDYYYGMDVWGQGTTVTVSSASTKGPSVFPLAPSSKSTSGGTAALGCLVKDYFPEPVTVSWNSGALTSGVHTFPAVLQSSGLYSLSSVVTVPSSSLGTQTYICNVNHKPSNTKVDKKVEPKSCDKTHTCPPCPAPEAAGGPSVFLFPPKPKDTLMISRTPEVTCVVVDVSHEDPEVKFNWYVDGVEVHNAKTKPREEQYNSTYRVVSVLTVLHQDWLNGKEYKCKVSNKALPAPIEKTISKAKGQPREPQVCTLPPSRDELTKNQVSLSCAVKGFYPSDIAVEWESNGQPENNYKTTPPVLDSDGSFFLVSKLTVDKSRWQQGNVFSCSVMHEALHNRFTQKSLSLSPG

SEQ ID NO: 60 - protein, 717 aa, Artificial Sequence
  anti-GITR-VL-huIGKC-[PCS2]-<(G4S)6>-[PCS2]-anti-GITR-VH-huIGHG1(LALA-hole-RF)
AIQLTQSPSSLSASVGDRVTITCRASQGISSALAWYQQKPGKAPKLLIYDASSLESGVPSRFSGSGSGTDFTLTISSLQPEDFATYYCQQFNSYPYTFGQGTKLEIKRTVAAPSVFIFPPSDEQLKSGTASVVCLLNNFYPREAKVQWKVDNALQSGNSQESVTEQDSKDSTYSLSSTLTLSKADYEKHKVYACEVTHQGLSSPVTKSFNRGECHRRRKRSVDEGGGGSGGGGSGGGGSGGGGSGGGGSGGGGSHRRRKRSVDEQVQLVESGGGVVQPGRSLRLSCAASGFTFSSYGMHWVRQAPGKGLEWVAVIWYEGSNKYYADSVKGRFTISRDNSKNTLYLQMNSLRAEDTAVYYCARGGSMVRGDYYYGMDVWGQGTTVTVSSASTKGPSVFPLAPSSKSTSGGTAALGCLVKDYFPEPVTVSWNSGALTSGVHTFPAVLQSSGLYSLSSVVTVPSSSLGTQTYICNVNHKPSNTKVDKKVEPKSCDKTHTCPPCPAPEAAGGPSVFLFPPKPKDTLMISRTPEVTCVVVDVSHEDPEVKFNWYVDGVEVHNAKTKPREEQYNSTYRVVSVLTVLHQDWLNGKEYKCKVSNKALPAPIEKTISKAKGQPREPQVCTLPPSRDELTKNQVSLSCAVKGFYPSDIAVEWESNGQPENNYKTTPPVLDSDGSFFLVSKLTVDKSRWQQGNVFSCSVMHEALHNRFTQKSLSLSPG

SEQ ID NO: 61 - protein, 717 aa, Artificial Sequence
  anti-GITR-VL-huIGKC-[PCS2a]-<(G4S)6>-[PCS2a]-anti-GITR-VH-huIGHG1(LALA-hole-RF)
AIQLTQSPSSLSASVGDRVTITCRASQGISSALAWYQQKPGKAPKLLIYDASSLESGVPSRFSGSGSGTDFTLTISSLQPEDFATYYCQQFNSYPYTFGQGTKLEIKRTVAAPSVFIFPPSDEQLKSGTASVVCLLNNFYPREAKVQWKVDNALQSGNSQESVTEQDSKDSTYSLSSTLTLSKADYEKHKVYACEVTHQGLSSPVTKSFNRGECHRRQQRSVDEGGGGSGGGGSGGGGSGGGGSGGGGSGGGGSHRRQQRSVDEQVQLVESGGGVVQPGRSLRLSCAASGFTFSSYGMHWVRQAPGKGLEWVAVIWYEGSNKYYADSVKGRFTISRDNSKNTLYLQMNSLRAEDTAVYYCARGGSMVRGDYYYGMDVWGQGTTVTVSSASTKGPSVFPLAPSSKSTSGGTAALGCLVKDYFPEPVTVSWNSGALTSGVHTFPAVLQSSGLYSLSSVVTVPSSSLGTQTYICNVNHKPSNTKVDKKVEPKSCDKTHTCPPCPAPEAAGGPSVFLFPPKPKDTLMISRTPEVTCVVVDVSHEDPEVKFNWYVDGVEVHNAKTKPREEQYNSTYRVVSVLTVLHQDWLNGKEYKCKVSNKALPAPIEKTISKAKGQPREPQVCTLPPSRDELTKNQVSLSCAVKGFYPSDIAVEWESNGQPENNYKTTPPVLDSDGSFFLVSKLTVDKSRWQQGNVFSCSVMHEALHNRFTQKSLSLSPG

SEQ ID NO: 62 - protein, 341 aa, Artificial Sequence
  anti-PD1-VL-<(G4S)2>-anti-GITR-VL-<(G4S)2>-huIGKC
EIVLTQSPATLSLSPGERATLSCRASQSVSSYLAWYQQKPGQAPRLLIYDASNRATGIPARFSGSGSGTDFTLTISSLEPEDFAVYYCQQSSNWPRTFGQGTKVEIKGGGGSGGGGSAIQLTQSPSSLSASVGDRVTITCRASQGISSALAWYQQKPGKAPKLLIYDASSLESGVPSRFSGSGSGTDFTLTISSLQPEDFATYYCQQFNSYPYTFGQGTKLEIKGGGGSGGGGSRTVAAPSVFIFPPSDEQLKSGTASVVCLLNNFYPREAKVQWKVDNALQSGNSQESVTEQDSKDSTYSLSSTLTLSKADYEKHKVYACEVTHQGLSSPVTKSFNRGEC

SEQ ID NO: 63 - protein, 566 aa, Artificial Sequence
  anti-GITR-VH-anti-PD1-VH-huIGHG1(LALA-knob)
QVQLVESGGGVVQPGRSLRLSCAASGFTFSSYGMHWVRQAPGKGLEWVAVIWYEGSNKYYADSVKGRFTISRDNSKNTLYLQMNSLRAEDTAVYYCARGGSMVRGDYYYGMDVWGQGTTVTVSSQVQLVESGGGVVQPGRSLRLDCKASGITFSNSGMHWVRQAPGKGLEWVAVIWYDGSKRYYADSVKGRFTISRDNSKNTLFLQMNSLRAEDTAVYYCATNDDYWGQGTLVTVSSASTKGPSVFPLAPSSKSTSGGTAALGCLVKDYFPEPVTVSWNSGALTSGVHTFPAVLQSSGLYSLSSVVTVPSSSLGTQTYICNVNHKPSNTKVDKKVEPKSCDKTHTCPPCPAPEAAGGPSVFLFPPKPKDTLMISRTPEVTCVVVDVSHEDPEVKFNWYVDGVEVHNAKTKPREEQYNSTYRVVSVLTVLHQDWLNGKEYKCKVSNKALPAPIEKTISKAKGQPREPQVYTLPPCRDELTKNQVSLWCLVKGFYPSDIAVEWESNGQPENNYKTTPPVLDSDGSFFLYSKLTVDKSRWQQGNVFSCSVMHEALHNHYTQKSLSLSPG

SEQ ID NO: 64 - protein, 710 aa, Artificial Sequence
  anti-OX40-VL-huIGKC-[PCS2]-<(G4S)6>-[PCS2]-anti-OX40-VH-huIGHG1(LALA-hole-RF)
DIQMTQSPSSLSASVGDRVTITCRASQDISNYLNWYQQKPGKAPKLLIYYTSRLRSGVPSRFSGSGSGTDFTLTISSLQPEDFATYYCQQGHTLPPTFGQGTKVEIKRTVAAPSVFIFPPSDEQLKSGTASVVCLLNNFYPREAKVQWKVDNALQSGNSQESVTEQDSKDSTYSLSSTLTLSKADYEKHKVYACEVTHQGLSSPVTKSFNRGECHRRRKRSVDEGGGGSGGGGSGGGGSGGGGSGGGGSGGGGSHRRRKRSVDEEVQLVQSGAEVKKPGASVKVSCKASGYTFTDSYMSWVRQAPGQGLEWIGDMYPDNGDSSYNQKFRERVTITRDTSTSTAYLELSSLRSEDTAVYYCVLAPRWYFSVWGQGTLVTVSSASTKGPSVFPLAPSSKSTSGGTAALGCLVKDYFPEPVTVSWNSGALTSGVHTFPAVLQSSGLYSLSSVVTVPSSSLGTQTYICNVNHKPSNTKVDKKVEPKSCDKTHTCPPCPAPEAAGGPSVFLFPPKPKDTLMISRTPEVTCVVVDVSHEDPEVKFNWYVDGVEVHNAKTKPREEQYNSTYRVVSVLTVLHQDWLNGKEYKCKVSNKALPAPIEKTISKAKGQPREPQVCTLPPSRDELTKNQVSLSCAVKGFYPSDIAVEWESNGQPENNYKTTPPVLDSDGSFFLVSKLTVDKSRWQQGNVFSCSVMHEALHNRFTQKSLSLSPG

SEQ ID NO: 65 - protein, 710 aa, Artificial Sequence
  anti-OX40-VL-huIGKC-[PCS2a]-<(G4S)6>-[PCS2a]-anti-OX40-VH-huIGHG1(LALA-hole-RF)
DIQMTQSPSSLSASVGDRVTITCRASQDISNYLNWYQQKPGKAPKLLIYYTSRLRSGVPSRFSGSGSGTDFTLTISSLQPEDFATYYCQQGHTLPPTFGQGTKVEIKRTVAAPSVFIFPPSDEQLKSGTASVVCLLNNFYPREAKVQWKVDNALQSGNSQESVTEQDSKDSTYSLSSTLTLSKADYEKHKVYACEVTHQGLSSPVTKSFNRGECHRRQQRSVDEGGGGSGGGGSGGGGSGGGGSGGGGSGGGGSHRRQQRSVDEEVQLVQSGAEVKKPGASVKVSCKASGYTFTDSYMSWVRQAPGQGLEWIGDMYPDNGDSSYNQKFRERVTITRDTSTSTAYLELSSLRSEDTAVYYCVLAPRWYFSVWGQGTLVTVSSASTKGPSVFPLAPSSKSTSGGTAALGCLVKDYFPEPVTVSWNSGALTSGVHTFPAVLQSSGLYSLSSVVTVPSSSLGTQTYICNVNHKPSNTKVDKKVEPKSCDKTHTCPPCPAPEAAGGPSVFLFPPKPKDTLMISRTPEVTCVVVDVSHEDPEVKFNWYVDGVEVHNAKTKPREEQYNSTYRVVSVLTVLHQDWLNGKEYKCKVSNKALPAPIEKTISKAKGQPREPQVCTLPPSRDELTKNQVSLSCAVKGFYPSDIAVEWESNGQPENNYKTTPPVLDSDGSFFLVSKLTVDKSRWQQGNVFSCSVMHEALHNRFTQKSLSLSPG

SEQ ID NO: 66 - protein, 341 aa, Artificial Sequence
  anti-GITR-VL-<(G4S)2>-anti-PD1-VL-<(G4S)2>-huIGKC
AIQLTQSPSSLSASVGDRVTITCRASQGISSALAWYQQKPGKAPKLLIYDASSLESGVPSRFSGSGSGTDFTLTISSLQPEDFATYYCQQFNSYPYTFGQGTKLEIKGGGGSGGGGSEIVLTQSPATLSLSPGERATLSCRASQSVSSYLAWYQQKPGQAPRLLIYDASNRATGIPARFSGSGSGTDFTLTISSLEPEDFAVYYCQQSSNWPRTFGQGTKVEIKGGGGSGGGGSRTVAAPSVFIFPPSDEQLKSGTASVVCLLNNFYPREAKVQWKVDNALQSGNSQESVTEQDSKDSTYSLSSTLTLSKADYEKHKVYACEVTHQGLSSPVTKSFNRGEC

SEQ ID NO: 67 - protein, 566 aa, Artificial Sequence
  anti-PD1-VH-anti-GITR-VH-huIGHG1(LALA-knob)
QVQLVESGGGVVQPGRSLRLDCKASGITFSNSGMHWVRQAPGKGLEWVAVIWYDGSKRYYADSVKGRFTISRDNSKNTLFLQMNSLRAEDTAVYYCATNDDYWGQGTLVTVSSQVQLVESGGGVVQPGRSLRLSCAASGFTFSSYGMHWVRQAPGKGLEWVAVIWYEGSNKYYADSVKGRFTISRDNSKNTLYLQMNSLRAEDTAVYYCARGGSMVRGDYYYGMDVWGQGTTVTVSSASTKGPSVFPLAPSSKSTSGGTAALGCLVKDYFPEPVTVSWNSGALTSGVHTFPAVLQSSGLYSLSSVVTVPSSSLGTQTYICNVNHKPSNTKVDKKVEPKSCDKTHTCPPCPAPEAAGGPSVFLFPPKPKDTLMISRTPEVTCVVVDVSHEDPEVKFNWYVDGVEVHNAKTKPREEQYNSTYRVVSVLTVLHQDWLNGKEYKCKVSNKALPAPIEKTISKAKGQPREPQVYTLPPCRDELTKNQVSLWCLVKGFYPSDIAVEWESNGQPENNYKTTPPVLDSDGSFFLYSKLTVDKSRWQQGNVFSCSVMHEALHNHYTQKSLSLSPG

SEQ ID NO: 68 - protein, 710 aa, Artificial Sequence; identical to SEQ ID NO: 64
  anti-OX40-VL-huIGKC-[PCS2]-<(G4S)6>-[PCS2]-anti-OX40-VH-huIGHG1(LALA-hole-RF)

SEQ ID NO: 69 - protein, 710 aa, Artificial Sequence; identical to SEQ ID NO: 65
  anti-OX40-VL-huIGKC-[PCS2a]-<(G4S)6>-[PCS2a]-anti-OX40-VH-huIGHG1(LALA-hole-RF)

SEQ ID NO: 70 - protein, 465 aa, Artificial Sequence
  anti-PD1-VL-huIGKC-[PCS2]-<(G4S)3>-[PCS2]-anti-4.1BB-VL-huIGKC
EIVLTQSPATLSLSPGERATLSCRASQSVSSYLAWYQQKPGQAPRLLIYDASNRATGIPARFSGSGSGTDFTLTISSLEPEDFAVYYCQQSSNWPRTFGQGTKVEIKRTVAAPSVFIFPPSDEQLKSGTASVVCLLNNFYPREAKVQWKVDNALQSGNSQESVTEQDSKDSTYSLSSTLTLSKADYEKHKVYACEVTHQGLSSPVTKSFNRGECHRRRKRSVDEGGGGSGGGGSGGGGSHRRRKRSVDEEIVLTQSPATLSLSPGERATLSCRASQSVSSYLAWYQQKPGQAPRLLIYDASNRATGIPARFSGSGSGTDFTLTISSLEPEDFAVYYCQQRSNWPPALTFGGGTKVEIKRTVAAPSVFIFPPSDEQLKSGTASVVCLLNNFYPREAKVQWKVDNALQSGNSQESVTEQDSKDSTYSLSSTLTLSKADYEKHKVYACEVTHQGLSSPVTKSFNRGEC

SEQ ID NO: 71 - protein, 686 aa, Artificial Sequence
  anti-PD1-VH-huIGH-G11-huIGH-H1-<(G4S)3>-anti-4.1BB-VH-huIGHG1-(LALA)
QVQLVESGGGVVQPGRSLRLDCKASGITFSNSGMHWVRQAPGKGLEWVAVIWYDGSKRYYADSVKGRFTISRDNSKNTLFLQMNSLRAEDTAVYYCATNDDYWGQGTLVTVSSASTKGPSVFPLAPSSKSTSGGTAALGCLVKDYFPEPVTVSWNSGALTSGVHTFPAVLQSSGLYSLSSVVTVPSSSLGTQTYICNVNHKPSNTKVDKKVEPKSCDKTHTGGGGSGGGGSGGGGSQVQLQQWGAGLLKPSETLSLTCAVYGGSFSGYYWSWIRQSPEKGLEWIGEINHGGYVTYNPSLESRVTISVDTSKNQFSLKLSSVTAADTAVYYCARDYGPGNYDWYFDLWGRGTLVTVSSASTKGPSVFPLAPSSKSTSGGTAALGCLVKDYFPEPVTVSWNSGALTSGVHTFPAVLQSSGLYSLSSVVTVPSSSLGTQTYICNVNHKPSNTKVDKKVEPKSCDKTHTCPPCPAPEAAGGPSVFLFPPKPKDTLMISRTPEVTCVVVDVSHEDPEVKFNWYVDGVEVHNAKTKPREEQYNSTYRVVSVLTVLHQDWLNGKEYKCKVSNKALPAPIEKTISKAKGQPREPQVYTLPPSRDELTKNQVSLTCLVKGFYPSDIAVEWESNGQPENNYKTTPPVLDSDGSFFLYSKLTVDKSRWQQGNVFSCSVMHEALHNHYTQKSLSLSPG

SEQ ID NO: 72 - protein, 465 aa, Artificial Sequence
  anti-PD1-VL-huIGKC-[PCS2a]-<(G4S)3>-[PCS2a]-anti-4.1BB-VL-huIGKC
EIVLTQSPATLSLSPGERATLSCRASQSVSSYLAWYQQKPGQAPRLLIYDASNRATGIPARFSGSGSGTDFTLTISSLEPEDFAVYYCQQSSNWPRTFGQGTKVEIKRTVAAPSVFIFPPSDEQLKSGTASVVCLLNNFYPREAKVQWKVDNALQSGNSQESVTEQDSKDSTYSLSSTLTLSKADYEKHKVYACEVTHQGLSSPVTKSFNRGECHRRQQRSVDEGGGGSGGGGSGGGGSHRRQQRSVDEEIVLTQSPATLSLSPGERATLSCRASQSVSSYLAWYQQKPGQAPRLLIYDASNRATGIPARFSGSGSGTDFTLTISSLEPEDFAVYYCQQRSNWPPALTFGGGTKVEIKRTVAAPSVFIFPPSDEQLKSGTASVVCLLNNFYPREAKVQWKVDNALQSGNSQESVTEQDSKDSTYSLSSTLTLSKADYEKHKVYACEVTHQGLSSPVTKSFNRGEC

SEQ ID NO: 73 - protein, 463 aa, Artificial Sequence
  anti-PD1-VL-huIGKC-[PCS2]-<(G4S)3>-[PCS2]-anti-OX40-VL-huIGKC
EIVLTQSPATLSLSPGERATLSCRASQSVSSYLAWYQQKPGQAPRLLIYDASNRATGIPARFSGSGSGTDFTLTISSLEPEDFAVYYCQQSSNWPRTFGQGTKVEIKRTVAAPSVFIFPPSDEQLKSGTASVVCLLNNFYPREAKVQWKVDNALQSGNSQESVTEQDSKDSTYSLSSTLTLSKADYEKHKVYACEVTHQGLSSPVTKSFNRGECHRRRKRSVDEGGGGSGGGGSGGGGSHRRRKRSVDEDIQMTQSPSSLSASVGDRVTITCRASQDISNYLNWYQQKPGKAPKLLIYYTSRLRSGVPSRFSGSGSGTDFTLTISSLQPEDFATYYCQQGHTLPPTFGQGTKVEIKRTVAAPSVFIFPPSDEQLKSGTASVVCLLNNFYPREAKVQWKVDNALQSGNSQESVTEQDSKDSTYSLSSTLTLSKADYEKHKVYACEVTHQGLSSPVTKSFNRGEC

SEQ ID NO: 74 - protein, 682 aa, Artificial Sequence
  anti-PD1-VH-huIGH-G11-huIGH-H1-<(G4S)3>-anti-OX40-VH-huIGHG1-(LALA)
QVQLVESGGGVVQPGRSLRLDCKASGITFSNSGMHWVRQAPGKGLEWVAVIWYDGSKRYYADSVKGRFTISRDNSKNTLFLQMNSLRAEDTAVYYCATNDDYWGQGTLVTVSSASTKGPSVFPLAPSSKSTSGGTAALGCLVKDYFPEPVTVSWNSGALTSGVHTFPAVLQSSGLYSLSSVVTVPSSSLGTQTYICNVNHKPSNTKVDKKVEPKSCDKTHTGGGGSGGGGSGGGGSEVQLVQSGAEVKKPGASVKVSCKASGYTFTDSYMSWVRQAPGQGLEWIGDMYPDNGDSSYNQKFRERVTITRDTSTSTAYLELSSLRSEDTAVYYCVLAPRWYFSVWGQGTLVTVSSASTKGPSVFPLAPSSKSTSGGTAALGCLVKDYFPEPVTVSWNSGALTSGVHTFPAVLQSSGLYSLSSVVTVPSSSLGTQTYICNVNHKPSNTKVDKKVEPKSCDKTHTCPPCPAPEAAGGPSVFLFPPKPKDTLMISRTPEVTCVVVDVSHEDPEVKFNWYVDGVEVHNAKTKPREEQYNSTYRVVSVLTVLHQDWLNGKEYKCKVSNKALPAPIEKTISKAKGQPREPQVYTLPPSRDELTKNQVSLTCLVKGFYPSDIAVEWESNGQPENNYKTTPPVLDSDGSFFLYSKLTVDKSRWQQGNVFSCSVMHEALHNHYTQKSLSLSPG

SEQ ID NO: 75 - protein, 463 aa, Artificial Sequence
  anti-PD1-VL-huIGKC-[PCS2a]-<(G4S)3>-[PCS2a]-anti-OX40-VL-huIGKC
EIVLTQSPATLSLSPGERATLSCRASQSVSSYLAWYQQKPGQAPRLLIYDASNRATGIPARFSGSGSGTDFTLTISSLEPEDFAVYYCQQSSNWPRTFGQGTKVEIKRTVAAPSVFIFPPSDEQLKSGTASVVCLLNNFYPREAKVQWKVDNALQSGNSQESVTEQDSKDSTYSLSSTLTLSKADYEKHKVYACEVTHQGLSSPVTKSFNRGECHRRQQRSVDEGGGGSGGGGSGGGGSHRRQQRSVDEDIQMTQSPSSLSASVGDRVTITCRASQDISNYLNWYQQKPGKAPKLLIYYTSRLRSGVPSRFSGSGSGTDFTLTISSLQPEDFATYYCQQGHTLPPTFGQGTKVEIKRTVAAPSVFIFPPSDEQLKSGTASVVCLLNNFYPREAKVQWKVDNALQSGNSQESVTEQDSKDSTYSLSSTLTLSKADYEKHKVYACEVTHQGLSSPVTKSFNRGEC